European Patent Specification EP 3 452 506 B1, published April 16, 2025. Title: AFFINITY ENGINEERED SERUM PROTEIN CARRIER BINDING DOMAIN. Applicant: UCB Biopharma SPRL. The sequence listing filed with the application follows.

SEQUENCE LISTING (9 sequences)

SEQ ID NO: 1 - protein, 118 aa, Artificial Sequence
  CA645 VH
QSLEESGGRLVTPGTPLTLTCTVSGIDLSNYAINWVRQAPGKGLEWIGIIWASGTTFYATWAKGRFTISRPSTTVDLEMTSLTTADTATYFCARTVPGYSTAPYFDLWGPGTLVTVSS

SEQ ID NO: 2 - protein, 119 aa, Artificial Sequence
  CA645 VH gH1
EVQLLESGGGLVQPGGSLRLSCAVSGIDLSNYAINWVRQAPGKGLEWIGIIWASGTTFYATWAKGRFTISRDSTTVYLQMNSLRAEDTAVYYCARTVPGYSTAPYFDLWGQGTLVTVSS

SEQ ID NO: 3 - protein, 121 aa, Artificial Sequence
  CA645 VH gH5
EVQLLESGGGLVQPGGSLRLSCAVSGIDLSNYAINWVRQAPGKGLEWIGIIWASGTTFYATWAKGRFTISRDNSKNTVYLQMNSLRAEDTAVYYCARTVPGYSTAPYFDLWGQGTLVTVSS

SEQ ID NO: 4 - protein, 121 aa, Artificial Sequence
  CA645 VH gH37
EVQLLESGGGLVQPGGSLRLSCAVSGIDLSNYAINWVRQAPGKGLEWIGIIWASGTTAYATWAKGRFTISRDNSKNTVYLQMNSLRAEDTAVYYCARTVPGYSTAPYFDLWGQGTLVTVSS

SEQ ID NO: 5 - protein, 121 aa, Artificial Sequence
  CA645 VH gH47
EVQLLESGGGLVQPGGSLRLSCAVSGIDLSNYAINWVRQAPGKGLEWIGIIWASGTTFYATWAKGRFTISRDNSKNTVYLQMNSLRAEDTAVYYCARTVPGYSAAPYFDLWGQGTLVTVSS

SEQ ID NO: 6 - protein, 110 aa, Artificial Sequence
  CA645 VL
AAVLTQTPSPVSAAVGGTVTINCQSSPSVWSNFLSWYQQKPGQPPKLLIYEASKLTSGVPSRFKGSGSGTQFTLTISDVQCGDAATYYCGGGYSSISDTTFGGGTKVVVK

SEQ ID NO: 7 - protein, 110 aa, Artificial Sequence
  CA645 VL gL1
DIVMTQSPSSVSASVGDRVTITCQSSPSVWSNFLSWYQQKPGKAPKLLIYEASKLTSGVPSRFKGSGSGTDFTLTISSLQPEDFATYYCGGGYSSISDTTFGGGTKVEIK

SEQ ID NO: 8 - protein, 110 aa, Artificial Sequence
  CA645 VL gL4
DIQMTQSPSSVSASVGDRVTITCQSSPSVWSNFLSWYQQKPGKAPKLLIYEASKLTSGVPSRFSGSGSGTDFTLTISSLQPEDFATYYCGGGYSSISDTTFGGGTKVEIK

SEQ ID NO: 9 - protein, 110 aa, Artificial Sequence
  CA645 VL gL5
DIQMTQSPSSVSASVGDRVTITCQSSPSVASNFLSWYQQKPGKAPKLLIYEASKLTSGVPSRFSGSGSGTDFTLTISSLQPEDFATYYCGGGYSSISDTTFGGGTKVEIK